European Patent Application EP 4 548 926 A1, published May 7, 2025. Title: γセクレターゼ阻害剤、Ａβペプチド産生抑制剤及び医薬. Applicant: 国立大学法人東北大学. The sequence listing filed with the application follows.

SEQUENCE LISTING (16 sequences)

SEQ ID NO: 1 - protein, 89 aa, Trimeresurus flavoviridis
MKTLLLILGVVAFVYLEPGYTRKCCIYPKSALFCREVQICPADEGMCFKMWNSTDRLMERTYVRGCAAACPNPVGDEEVYCCVTDNCNK

SEQ ID NO: 2 - protein, 85 aa, Trimeresurus flavoviridis
MKTLLLILGVVAFVYLDSGFSLICNTCNRTVRIPLIPCDPVTCPEGLDQCYANRTGILRMKVERGCTTNCTQTLTLMCCKRDMCN

SEQ ID NO: 3 - protein, 85 aa, Trimeresurus flavoviridis
MKTHLLALVMVAFLYLEPGYTLRCHSCVGYVCKEFEFCKPEQKQCIYLINRKKYSGCSRNCPSAGANELVKCCATDRCNLEIFCW

SEQ ID NO: 4 - protein, 82 aa, Trimeresurus flavoviridis
MKTLLLILGVVAFVYLDSGFSLKCEQCNLPNCDFLPDVRCPKGLDQCYKKWNETAKVFERGCTANCNEDEQTRCCKRNGCNF

SEQ ID NO: 5 - DNA, 36 bp, synthetic construct
  source 1..36: mol_type = other DNA
cttgttctttacgaccatcatcatcatcatcatatg

SEQ ID NO: 6 - DNA, 33 bp, synthetic construct
  source 1..33: mol_type = other DNA
gactctagaggatccgaattcggatccctcgag

SEQ ID NO: 7 - DNA, 23 bp, synthetic construct
  source 1..23: mol_type = other DNA
gtcgtaaagaacaagcgttcttg

SEQ ID NO: 8 - DNA, 22 bp, synthetic construct
  source 1..22: mol_type = other DNA
ggatcctctagagtcgacctgc

SEQ ID NO: 9 - DNA, 43 bp, synthetic construct
  source 1..43: mol_type = other DNA
cacaaagtgcatcatcatcatcatcatatggtgagcaagggcg

SEQ ID NO: 10 - DNA, 31 bp, synthetic construct
  source 1..31: mol_type = other DNA
atgcctaccttcgatgtacagctcgtccatg

SEQ ID NO: 11 - DNA, 18 bp, synthetic construct
  source 1..18: mol_type = other DNA
atcgaaggtaggcatatg

SEQ ID NO: 12 - DNA, 31 bp, synthetic construct
  source 1..31: mol_type = other DNA
atgatgatgatgatgatgcactttgtgattc

SEQ ID NO: 13 - DNA, 29 bp, synthetic construct
  source 1..29: mol_type = other DNA
ccccgatcctatatgatgcttttgcaagc

SEQ ID NO: 14 - DNA, 22 bp, synthetic construct
  source 1..22: mol_type = other DNA
tagcttcatactagtgccatgc

SEQ ID NO: 15 - DNA, 23 bp, synthetic construct
  source 1..23: mol_type = other DNA
actagtatgaagctactgtcttc

SEQ ID NO: 16 - DNA, 24 bp, synthetic construct
  source 1..24: mol_type = other DNA
catataggatcggggagttgattg